European Patent Specification EP 3 311 168 B1, published May 10, 2023. Title: NOVEL TNFA STRUCTURE FOR USE IN THERAPY. Applicant: UCB Biopharma SPRL. The sequence listing filed with the application follows.

SEQUENCE LISTING (36 sequences)

SEQ ID NO: 1 - protein, 8 aa, Artificial Sequence
  LCDR1 of 1974/1979
QASQDIGN

SEQ ID NO: 2 - protein, 7 aa, Artificial Sequence
  LCDR2 of 1974
GATSLAD

SEQ ID NO: 3 - protein, 9 aa, Artificial Sequence
  LCDR3 of 1974
LQGQSTPYT

SEQ ID NO: 4 - protein, 5 aa, Artificial Sequence
  HCDR1 of 1974
AYYMA

SEQ ID NO: 5 - protein, 18 aa, Artificial Sequence
  HCDR2 of 1974
ASINYDGANTFYRDSVKG

SEQ ID NO: 6 - protein, 12 aa, Artificial Sequence
  HCDR3 of 1974
EAYGYNSNWFGY

SEQ ID NO: 7 - protein, 107 aa, Artificial Sequence
  LCVR of 1974
DIQMTQSPASLPASPEEIVTITCQASQDIGNWLSWYQQKPGKSPQLLIYGATSLADGVPSRFSASRSGTQYSLKISRLQVEDFGIFYCLQGQSTPYTFGAGTKLELK

SEQ ID NO: 8 - protein, 121 aa, Artificial Sequence
  HCVR of 1974
DVQLVESGGGLVQPGRSLKLSCAASGFTFSAYYMAWVRQAPTKGLEWVASINYDGANTFYRDSVKGRFTVSRDNARSSLYLQMDSLRSEDTATYYCTTEAYGYNSNWFGYWGQGTLVTVSS

SEQ ID NO: 9 - DNA, 321 bp, Artificial Sequence
  LCVR DNA of 1974
gacatccagatgacccagtctcctgcctccctgcctgcatccccggaagaaattgtcaccatcacatgccaggcaagccaggacattggtaattggttatcatggtatcagcagaaaccagggaaatcgcctcagctcctgatctatggtgcaaccagcttggcagatggggtcccatcaaggttcagcgccagtagatctggcacacagtactctcttaagatcagcagactgcaggttgaagattttggaatcttttactgtctacagggtcaaagtactccgtacacgtttggagctgggaccaagctggaactgaaa

SEQ ID NO: 10 - DNA, 363 bp, Artificial Sequence
  HCVR DNA of 1974
gacgtgcagctggtggaatctggaggaggcttagtgcagcctggaaggtccctgaaactctcctgtgcagcctcaggattcactttcagtgcctattacatggcctgggtccgccaggctccaacgaagggtctggagtgggtcgcatccattaattatgatggtgctaacactttctatcgcgactccgtgaagggccgattcactgtctccagagataatgcaagaagcagcctatacctacaaatggacagtctgaggtctgaggacacggccacttattactgtacaacagaggcttacggatataactcaaattggtttggttactggggccaaggcactctggtcactgtctcgagc

SEQ ID NO: 11 - protein, 214 aa, Artificial Sequence
  1974 LC kappa full
DIQMTQSPASLPASPEEIVTITCQASQDIGNWLSWYQQKPGKSPQLLIYGATSLADGVPSRFSASRSGTQYSLKISRLQVEDFGIFYCLQGQSTPYTFGAGTKLELKRTDAAPTVSIFPPSSEQLTSGGASVVCFLNNFYPKDINVKWKIDGSERQNGVLNSWTDQDSKDSTYSMSSTLTLTKDEYERHNSYTCEATHKTSTSPIVKSFNRNEC

SEQ ID NO: 12 - protein, 445 aa, Artificial Sequence
  1974 HC mIgG1 full
DVQLVESGGGLVQPGRSLKLSCAASGFTFSAYYMAWVRQAPTKGLEWVASINYDGANTFYRDSVKGRFTVSRDNARSSLYLQMDSLRSEDTATYYCTTEAYGYNSNWFGYWGQGTLVTVSSAKTTPPSVYPLAPGSAAQTNSMVTLGCLVKGYFPEPVTVTWNSGSLSSGVHTFPAVLQSDLYTLSSSVTVPSSTWPSETVTCNVAHPASSTKVDKKIVPRDCGCKPCICTVPEVSSVFIFPPKPKDVLTITLTPKVTCVVVDISKDDPEVQFSWFVDDVEVHTAQTQPREEQFNSTFRSVSELPIMHQDWLNGKEFKCRVNSAAFPAPIEKTISKTKGRPKAPQVYTIPPPKEQMAKDKVSLTCMITDFFPEDITVEWQWNGQPAENYKNTQPIMDTDGSYFVYSKLNVQKSNWEAGNTFTCSVLHEGLHNHHTEKSLSHSPGK

SEQ ID NO: 13 - protein, 223 aa, Artificial Sequence
  1974 HC mFabno hinge full
DVQLVESGGGLVQPGRSLKLSCAASGFTFSAYYMAWVRQAPTKGLEWVASINYDGANTFYRDSVKGRFTVSRDNARSSLYLQMDSLRSEDTATYYCTTEAYGYNSNWFGYWGQGTLVTVSSAKTTPPSVYPLAPGSAAQTNSMVTLGCLVKGYFPEPVTVTWNSGSLSSGVHTFPAVLQSDLYTLSSSVTVPSSTWPSETVTCNVAHPASSTKVDKKIVPRDC

SEQ ID NO: 14 - DNA, 642 bp, Artificial Sequence
  1974 LC DNA kappa full
gacatccagatgacccagtctcctgcctccctgcctgcatccccggaagaaattgtcaccatcacatgccaggcaagccaggacattggtaattggttatcatggtatcagcagaaaccagggaaatcgcctcagctcctgatctatggtgcaaccagcttggcagatggggtcccatcaaggttcagcgccagtagatctggcacacagtactctcttaagatcagcagactgcaggttgaagattttggaatcttttactgtctacagggtcaaagtactccgtacacgtttggagctgggaccaagctggaactgaaacgtacggatgctgcaccaactgtatccatcttcccaccatccagtgagcagttaacatctggaggtgcctcagtcgtgtgcttcttgaacaacttctaccccaaagacatcaatgtcaagtggaagattgatggcagtgaacgacaaaatggcgtcctgaacagttggactgatcaggacagcaaagacagcacctacagcatgagcagcaccctcacgttgaccaaggacgagtatgaacgacataacagctatacctgtgaggccactcacaagacatcaacttcacccattgtcaagagcttcaacaggaatgagtgt

SEQ ID NO: 15 - DNA, 1335 bp, Artificial Sequence
  1974 HC DNA mIgG1 full
gacgtgcagctggtggaatctggaggaggcttagtgcagcctggaaggtccctgaaactctcctgtgcagcctcaggattcactttcagtgcctattacatggcctgggtccgccaggctccaacgaagggtctggagtgggtcgcatccattaattatgatggtgctaacactttctatcgcgactccgtgaagggccgattcactgtctccagagataatgcaagaagcagcctatacctacaaatggacagtctgaggtctgaggacacggccacttattactgtacaacagaggcttacggatataactcaaattggtttggttactggggccaaggcactctggtcactgtctcgagtgccaaaacgacacccccatctgtctatccactggcccctggatctgctgcccaaactaactccatggtgaccctgggatgcctggtcaagggctatttccctgagccagtgacagtgacctggaactctggatccctgtccagcggtgtgcacaccttcccagctgtcctgcagtctgacctctacactctgagcagctcagtgactgtcccctccagcacctggcccagcgagaccgtcacctgcaacgttgcccacccggccagcagcaccaaggtggacaagaaaattgtgcccagggattgtggttgtaagccttgcatatgtacagtcccagaagtatcatctgtcttcatcttccccccaaagcccaaggatgtgctcaccattactctgactcctaaggtcacgtgtgttgtggtagacatcagcaaggatgatcccgaggtccagttcagctggtttgtagatgatgtggaggtgcacacagctcagacgcaaccccgggaggagcagttcaacagcactttccgctcagtcagtgaacttcccatcatgcaccaggactggctcaatggcaaggagttcaaatgcagggtcaacagtgcagctttccctgcccccatcgagaaaaccatctccaaaaccaaaggcagaccgaaggctccacaggtgtacaccattccacctcccaaggagcagatggccaaggataaagtcagtctgacctgcatgataacagacttcttccctgaagacattactgtggagtggcagtggaatgggcagccagcggagaactacaagaacactcagcccatcatggacacagatggctcttacttcgtctacagcaagctcaatgtgcagaagagcaactgggaggcaggaaatactttcacctgctctgtgttacatgagggcctgcacaaccaccatactgagaagagcctctcccactctcctggtaaa

SEQ ID NO: 16 - DNA, 669 bp, Artificial Sequence
  1974 HC DNA mFabno hinge full
gacgtgcagctggtggaatctggaggaggcttagtgcagcctggaaggtccctgaaactctcctgtgcagcctcaggattcactttcagtgcctattacatggcctgggtccgccaggctccaacgaagggtctggagtgggtcgcatccattaattatgatggtgctaacactttctatcgcgactccgtgaagggccgattcactgtctccagagataatgcaagaagcagcctatacctacaaatggacagtctgaggtctgaggacacggccacttattactgtacaacagaggcttacggatataactcaaattggtttggttactggggccaaggcactctggtcactgtctcgagtgccaaaacgacacccccatctgtctatccactggcccctggatctgctgcccaaactaactccatggtgaccctgggatgcctggtcaagggctatttccctgagccagtgacagtgacctggaactctggatccctgtccagcggtgtgcacaccttcccggctgtcctgcaatctgacctctacactctgagcagctcagtgactgtcccctccagcacctggcccagcgagaccgtcacctgcaacgttgcccacccggccagcagcaccaaggtggacaagaaaattgtgcccagggattgt

SEQ ID NO: 17 - protein, 7 aa, Artificial Sequence
  LCDR2 of 1979
GTTSLAD

SEQ ID NO: 18 - protein, 10 aa, Artificial Sequence
  LCDR3 of 1979
LQAYSTPFTF

SEQ ID NO: 19 - protein, 5 aa, Artificial Sequence
  HCDR1 of 1979
NSYWD

SEQ ID NO: 20 - protein, 16 aa, Artificial Sequence
  HCDR2 of 1979
YINYSGSTGYNPSLKS

SEQ ID NO: 21 - protein, 12 aa, Artificial Sequence
  HCDR3 of 1979
GTYGYNAYHFDY

SEQ ID NO: 22 - protein, 107 aa, Artificial Sequence
  LCVR 1979
DIQMTQSPASLSASLEEIVTITCQASQDIGNWLSWYQQKPGKSPHLLIYGTTSLADGVPSRFSGSRSGTQYSLKISGLQVADIGIYVCLQAYSTPFTFGSGTKLEIK

SEQ ID NO: 23 - protein, 120 aa, Artificial Sequence
  HCVR of 1979
EVHLVESGPGLVKPSQSLSLTCSVTGYSITNSYWDWIRKFPGNKMEWMGYINYSGSTGYNPSLKSRISISRDTSNNQFFLQLNSITTEDTATYYCARGTYGYNAYHFDYWGRGVMVTVSS

SEQ ID NO: 24 - DNA, 321 bp, Artificial Sequence
  LCVR DNA of 1979
gacatccaaatgacacagtctcctgcctccctgtctgcatctctggaagaaattgtcaccattacatgccaggcaagccaggacattggtaattggttatcatggtatcagcagaaaccagggaaatctcctcacctcctgatctatggtaccaccagcttggcagatggggtcccatcaaggttcagcggcagtagatctggtacacagtattctcttaagatcagcggactacaggttgcagatattggaatctatgtctgtctacaggcttatagtactccattcacgttcggctcagggacaaagctggaaataaaa

SEQ ID NO: 25 - DNA, 360 bp, Artificial Sequence
  HCVR DNA of 1979
gaggtgcacctggtggagtctggacctggccttgtgaaaccctcacagtcactctccctcacctgttctgtcactggttactccatcactaatagttactgggactggatccggaagttcccaggaaataaaatggagtggatgggatacataaactacagtggtagcactggctacaacccatctctcaaaagtcgaatctccattagtagagacacatcgaacaatcagttcttcctgcagctgaactctataactactgaggacacagccacatattactgtgcacgagggacctatgggtataacgcctaccactttgattactggggccgaggagtcatggtcacagtctcgagc

SEQ ID NO: 26 - protein, 214 aa, Artificial Sequence
  1979 LC Kappa full
DIQMTQSPASLSASLEEIVTITCQASQDIGNWLSWYQQKPGKSPHLLIYGTTSLADGVPSRFSGSRSGTQYSLKISGLQVADIGIYVCLQAYSTPFTFGSGTKLEIKRTDAAPTVSIFPPSSEQLTSGGASVVCFLNNFYPKDINVKWKIDGSERQNGVLNSWTDQDSKDSTYSMSSTLTLTKDEYERHNSYTCEATHKTSTSPIVKSFNRNEC

SEQ ID NO: 27 - protein, 444 aa, Artificial Sequence
  1979 HC mIgG1 full
EVHLVESGPGLVKPSQSLSLTCSVTGYSITNSYWDWIRKFPGNKMEWMGYINYSGSTGYNPSLKSRISISRDTSNNQFFLQLNSITTEDTATYYCARGTYGYNAYHFDYWGRGVMVTVSSAKTTPPSVYPLAPGSAAQTNSMVTLGCLVKGYFPEPVTVTWNSGSLSSGVHTFPAVLQSDLYTLSSSVTVPSSTWPSETVTCNVAHPASSTKVDKKIVPRDCGCKPCICTVPEVSSVFIFPPKPKDVLTITLTPKVTCVVVDISKDDPEVQFSWFVDDVEVHTAQTQPREEQFNSTFRSVSELPIMHQDWLNGKEFKCRVNSAAFPAPIEKTISKTKGRPKAPQVYTIPPPKEQMAKDKVSLTCMITDFFPEDITVEWQWNGQPAENYKNTQPIMDTDGSYFVYSKLNVQKSNWEAGNTFTCSVLHEGLHNHHTEKSLSHSPGK

SEQ ID NO: 28 - protein, 222 aa, Artificial Sequence
  1979 HC mFabno hinge full
EVHLVESGPGLVKPSQSLSLTCSVTGYSITNSYWDWIRKFPGNKMEWMGYINYSGSTGYNPSLKSRISISRDTSNNQFFLQLNSITTEDTATYYCARGTYGYNAYHFDYWGRGVMVTVSSAKTTPPSVYPLAPGSAAQTNSMVTLGCLVKGYFPEPVTVTWNSGSLSSGVHTFPAVLQSDLYTLSSSVTVPSSTWPSETVTCNVAHPASSTKVDKKIVPRDC

SEQ ID NO: 29 - DNA, 642 bp, Artificial Sequence
  1979 LC DNA Kappa full
gacatccaaatgacacagtctcctgcctccctgtctgcatctctggaagaaattgtcaccattacatgccaggcaagccaggacattggtaattggttatcatggtatcagcagaaaccagggaaatctcctcacctcctgatctatggtaccaccagcttggcagatggggtcccatcaaggttcagcggcagtagatctggtacacagtattctcttaagatcagcggactacaggttgcagatattggaatctatgtctgtctacaggcttatagtactccattcacgttcggctcagggacaaagctggaaataaaacgtacggatgctgcaccaactgtatccatcttcccaccatccagtgagcagttaacatctggaggtgcctcagtcgtgtgcttcttgaacaacttctaccccaaagacatcaatgtcaagtggaagattgatggcagtgaacgacaaaatggcgtcctgaacagttggactgatcaggacagcaaagacagcacctacagcatgagcagcaccctcacgttgaccaaggacgagtatgaacgacataacagctatacctgtgaggccactcacaagacatcaacttcacccattgtcaagagcttcaacaggaatgagtgt

SEQ ID NO: 30 - DNA, 1332 bp, Artificial Sequence
  1979 HC DNA mIgG1 full
gaggtgcacctggtggagtctggacctggccttgtgaaaccctcacagtcactctccctcacctgttctgtcactggttactccatcactaatagttactgggactggatccggaagttcccaggaaataaaatggagtggatgggatacataaactacagtggtagcactggctacaacccatctctcaaaagtcgaatctccattagtagagacacatcgaacaatcagttcttcctgcagctgaactctataactactgaggacacagccacatattactgtgcacgagggacctatgggtataacgcctaccactttgattactggggccgaggagtcatggtcacagtctcgagtgccaaaacgacacccccatctgtctatccactggcccctggatctgctgcccaaactaactccatggtgaccctgggatgcctggtcaagggctatttccctgagccagtgacagtgacctggaactctggatccctgtccagcggtgtgcacaccttcccagctgtcctgcagtctgacctctacactctgagcagctcagtgactgtcccctccagcacctggcccagcgagaccgtcacctgcaacgttgcccacccggccagcagcaccaaggtggacaagaaaattgtgcccagggattgtggttgtaagccttgcatatgtacagtcccagaagtatcatctgtcttcatcttccccccaaagcccaaggatgtgctcaccattactctgactcctaaggtcacgtgtgttgtggtagacatcagcaaggatgatcccgaggtccagttcagctggtttgtagatgatgtggaggtgcacacagctcagacgcaaccccgggaggagcagttcaacagcactttccgctcagtcagtgaacttcccatcatgcaccaggactggctcaatggcaaggagttcaaatgcagggtcaacagtgcagctttccctgcccccatcgagaaaaccatctccaaaaccaaaggcagaccgaaggctccacaggtgtacaccattccacctcccaaggagcagatggccaaggataaagtcagtctgacctgcatgataacagacttcttccctgaagacattactgtggagtggcagtggaatgggcagccagcggagaactacaagaacactcagcccatcatggacacagatggctcttacttcgtctacagcaagctcaatgtgcagaagagcaactgggaggcaggaaatactttcacctgctctgtgttacatgagggcctgcacaaccaccatactgagaagagcctctcccactctcctggtaaa

SEQ ID NO: 31 - DNA, 666 bp, Artificial Sequence
  1979 HC DNA mFabno hinge full
gaggtgcacctggtggagtctggacctggccttgtgaaaccctcacagtcactctccctcacctgttctgtcactggttactccatcactaatagttactgggactggatccggaagttcccaggaaataaaatggagtggatgggatacataaactacagtggtagcactggctacaacccatctctcaaaagtcgaatctccattagtagagacacatcgaacaatcagttcttcctgcagctgaactctataactactgaggacacagccacatattactgtgcacgagggacctatgggtataacgcctaccactttgattactggggccgaggagtcatggtcacagtctcgagtgccaaaacgacacccccatctgtctatccactggcccctggatctgctgcccaaactaactccatggtgaccctgggatgcctggtcaagggctatttccctgagccagtgacagtgacctggaactctggatccctgtccagcggtgtgcacaccttcccggctgtcctgcaatctgacctctacactctgagcagctcagtgactgtcccctccagcacctggcccagcgagaccgtcacctgcaacgttgcccacccggccagcagcaccaaggtggacaagaaaattgtgcccagggattgt

SEQ ID NO: 32 - protein, 235 aa, Rattus norvegicus
MSTESMIRDVELAEEALPKKMGGLQNSRRCLCLSLFSFLLVAGATTLFCLLNFGVIGPNKEEKFPNGLPLISSMAQTLTLRSSSQNSSDKPVAHVVANHQAEEQLEWLSQRANALLANGMDLKDNQLVVPADGLYLIYSQVLFKGQGCPDYVLLTHTVSRFAISYQEKVSLLSAIKSPCPKDTPEGAELKPWYEPMYLGGVFQLEKGDLLSAEVNLPKYLDITESGQVYFGVIAL

SEQ ID NO: 33 - protein, 235 aa, Mus musculus
MSTESMIRDVELAEEALPQKMGGFQNSRRCLCLSLFSFLLVAGATTLFCLLNFGVIGPQRDEKFPNGLPLISSMAQTLTLRSSSQNSSDKPVAHVVANHQVEEQLEWLSQRANALLANGMDLKDNQLVVPADGLYLVYSQVLFKGQGCPDYVLLTHTVSRFAISYQEKVNLLSAVKSPCPKDTPEGAELKPWYEPIYLGGVFQLEKGDQLSAEVNLPKYLDFAESGQVYFGVIAL

SEQ ID NO: 34 - protein, 233 aa, Homo sapiens
MSTESMIRDVELAEEALPKKTGGPQGSRRCLFLSLFSFLIVAGATTLFCLLHFGVIGPQREEFPRDLSLISPLAQAVRSSSRTPSDKPVAHVVANPQAEGQLQWLNRRANALLANGVELRDNQLVVPSEGLYLIYSQVLFKGQGCPSTHVLLTHTISRIAVSYQTKVNLLSAIKSPCQRETPEGAEAKPWYEPIYLGGVFQLEKGDRLSAEINRPDYLDFAESGQVYFGIIAL

SEQ ID NO: 35 - protein, 158 aa, Homo sapiens
SVRSSSRTPSDKPVAHVVANPQAEGQLQWLNRRANALLANGVELRDNQLVVPSEGLYLIYSQVLFKGQGCPSTHVLLTHTISRIAVSYQTKVNLLSAIKSPCQRETPEGAEAKPWYEPIYLGGVFQLEKGDRLSAEINRPDYLDFAESGQVYFGIIAL

SEQ ID NO: 36 - protein, 157 aa, Homo sapiens [sequence omitted]